European Patent Specification EP 3 516 400 B1, published August 16, 2023. Title: MEASUREMENT OF PROTEIN EXPRESSION USING REAGENTS WITH BARCODED OLIGONUCLEOTIDE SEQUENCES. Applicant: Cellular Research, Inc. Becton, Dickinson and Company Fan, Christina Chang, Christina Shum, Eleen Zoellner, Olaf Bansal, Nidhanjali Ghadiali, James Lam, Gretchen Yinbon Jensen, Eric Rohrer, Jurg Gaylord, Brent Martin, Jody Vidal, Jason G. The sequence listing filed with the application follows.

SEQUENCE LISTING (7 sequences)

SEQ ID NO: 1 - DNA, 20 bp, Artificial Sequence
  note="Description of Artificial Sequence: Synthetic Oligonucleotide"
aaaaaaaaaaaaaaaaaaaa

SEQ ID NO: 2 - DNA, 20 bp, Artificial Sequence
  note="Description of Artificial Sequence: Synthetic Oligonucleotide"
tttttttttttttttttttt

SEQ ID NO: 3 - DNA, 95 bp, Artificial Sequence
  note="Description of Artificial Sequence: Synthetic Oligonucleotide"
  5AmMC6 (1)..(1): 5' Amino Modifier C6
gttgtcaagatgctaccgttcagagtacgtggagttggtggcccgaccccgagcgctacgagccccccggaaaaaaaaaaaaaaaaaaaaaaaaa

SEQ ID NO: 4 - DNA, 200 bp, Artificial Sequence
  note="Description of Artificial Sequence: Synthetic Oligonucleotide"
  5AmMC6 (1)..(1): 5' Amino Modifier C6
gttgtcaagatgctaccgttcagagctactgtccgaagttaccgtgtatctaccacgggtggtttttcgaatccggaaaagatagtaataagtgttttagttggaataagtcgcaacttttggagacggttacctctcaatttttctgatccgtaggccccccgatctcggcctcaaaaaaaaaaaaaaaaaaaaaaaaa

SEQ ID NO: 5 - DNA, 25 bp, Artificial Sequence
  note="Description of Artificial Sequence: Synthetic Oligonucleotide"
gttgtcaagatgctaccgttcagag

SEQ ID NO: 6 - DNA, 95 bp, Artificial Sequence
  note="Description of Artificial Sequence: Synthetic Oligonucleotide"
gttgtcaagatgctaccgttcagagccccatgtctagtacctattggtcccctatcctcagattcgtttaaaaaaaaaaaaaaaaaaaaaaaaaa

SEQ ID NO: 7 - DNA, 26 bp, Artificial Sequence
  note="Description of Artificial Sequence: Synthetic Oligonucleotide"
tttttttttttttttttttttttttt